European Patent Specification EP 3 556 855 B1, published January 14, 2026. Title: GENE-MODIFIED LYMPHOCYTES EXPRESSING CHIMERIC ANTIGEN RECEPTOR. Applicant: SHINSHU UNIVERSITY KYOTO PREFECTURAL PUBLIC UNIVERSITY CORPORATION. The sequence listing filed with the application follows.

SEQUENCE LISTING (10 sequences)

SEQ ID NO: 1 - protein, 227 aa, Homo sapiens
MAVRRDSVWKYCWGVLMVLCRTAISKSIVLEPIYWNSSNSKFLPGQGLVLYPQIGDKLDIICPKVDSKTVGQYEYYKVYMVDKDQADRCTIKKENTPLLNCAKPDQDIKFTIKFQEFSPNLWGLEFQKNKDYYIISTSNGSLEGLDNQEGGVCQTRAMKILMKVGQDASSAGSTRNKDPTRRPELEAGTNGRSSTTSPFVKPNPGSSTDGNSAGHSGNNILGSEVAL

SEQ ID NO: 2 - protein, 333 aa, Homo sapiens
MAVRRDSVWKYCWGVLMVLCRTAISKSIVLEPIYWNSSNSKFLPGQGLVLYPQIGDKLDIICPKVDSKTVGQYEYYKVYMVDKDQADRCTIKKENTPLLNCAKPDQDIKFTIKFQEFSPNLWGLEFQKNKDYYIISTSNGSLEGLDNQEGGVCQTRAMKILMKVGQDASSAGSTRNKDPTRRPELEAGTNGRSSTTSPFVKPNPGSSTDGNSAGHSGNNILGSEVALFAGIASGCIIFIVIIITLVVLLLKYRRRHRKHSPQHTTTLSLSTLATPKRSGNNNGSEPSDIIIPLRTADSVFCPHYEKVSGDYGHPVYIVQEMPPQSPANIYYKV

SEQ ID NO: 3 - DNA, 1356 bp, Artificial Sequence
  EPHB4-CAR gene
atggctgtgagaagggactccgtgtggaagtactgctggggtgttttgatggttttatgcagaactgcgatttccaaatcgatagttttagagcctatctattggaattcctcgaactccaaatttctacctggacaaggactggtactatacccacagataggagacaaattggatattatttgccccaaagtggactctaaaactgttggccagtatgaatattataaagtttatatggttgataaagaccaagcagacagatgcactattaagaaggaaaatacccctctcctcaactgtgccaaaccagaccaagatatcaaattcaccatcaagtttcaagaattcagccctaacctctggggtctagaatttcagaagaacaaagattattacattatatctacatcaaatgggtctttggagggcctggataaccaggagggaggggtgtgccagacaagagccatgaagatcctcatgaaagttggacaagatgcaagttctgctggatcaaccaggaataaagatccaacaagacgtccagaactagaagctggtacaaatggaagaagttcgacaacaagtccctttgtaaaaccaaatccaggttctagcacagacggcaacagcgccggacattcggggaacaacatcctcggttccgaagtggccttatcctcagcggccgcaattgaagttatgtatcctcctccttacctagacaatgagaagagcaatggaaccattatccatgtgaaagggaaacacctttgtccaagtcccctatttcccggaccttctaagcccttttgggtgctggtggtggttgggggagtcctggcttgctatagcttgctagtaacagtggcctttattattttctgggtgaggagtaagaggagcaggctcctgcacagtgactacatgaacatgactccccgccgccccgggcccacccgcaagcattaccagccctatgccccaccacgcgacttcgcagcctatcgctccagagtgaagttcagcaggagcgcagacgcccccgcgtaccagcagggccagaaccagctctataacgagctcaatctaggacgaagagaggagtacgatgttttggacaagagacgtggccgggaccctgagatggggggaaagccgagaaggaagaaccctcaggaaggcctgtacaatgaactgcagaaagataagatggcggaggcctacagtgagattgggatgaaaggcgagcgccggaggggcaaggggcacgatggcctttaccagggtctcagtacagccaccaaggacacctacgacgcccttcacatgcaggccctgccccctcgctaa

SEQ ID NO: 4 - DNA, 5660 bp, Artificial Sequence
  pIRII-EPHB4-CAR vector
tcgagatggctgtgagaagggactccgtgtggaagtactgctggggtgttttgatggttttatgcagaactgcgatttccaaatcgatagttttagagcctatctattggaattcctcgaactccaaatttctacctggacaaggactggtactatacccacagataggagacaaattggatattatttgccccaaagtggactctaaaactgttggccagtatgaatattataaagtttatatggttgataaagaccaagcagacagatgcactattaagaaggaaaatacccctctcctcaactgtgccaaaccagaccaagatatcaaattcaccatcaagtttcaagaattcagccctaacctctggggtctagaatttcagaagaacaaagattattacattatatctacatcaaatgggtctttggagggcctggataaccaggagggaggggtgtgccagacaagagccatgaagatcctcatgaaagttggacaagatgcaagttctgctggatcaaccaggaataaagatccaacaagacgtccagaactagaagctggtacaaatggaagaagttcgacaacaagtccctttgtaaaaccaaatccaggttctagcacagacggcaacagcgccggacattcggggaacaacatcctcggttccgaagtggccttatcctcagcggccgcaattgaagttatgtatcctcctccttacctagacaatgagaagagcaatggaaccattatccatgtgaaagggaaacacctttgtccaagtcccctatttcccggaccttctaagcccttttgggtgctggtggtggttgggggagtcctggcttgctatagcttgctagtaacagtggcctttattattttctgggtgaggagtaagaggagcaggctcctgcacagtgactacatgaacatgactccccgccgccccgggcccacccgcaagcattaccagccctatgccccaccacgcgacttcgcagcctatcgctccagagtgaagttcagcaggagcgcagacgcccccgcgtaccagcagggccagaaccagctctataacgagctcaatctaggacgaagagaggagtacgatgttttggacaagagacgtggccgggaccctgagatggggggaaagccgagaaggaagaaccctcaggaaggcctgtacaatgaactgcagaaagataagatggcggaggcctacagtgagattgggatgaaaggcgagcgccggaggggcaaggggcacgatggcctttaccagggtctcagtacagccaccaaggacacctacgacgcccttcacatgcaggccctgccccctcgctaaggtaccggttgttaacgttagccggctacgtatactccggaatattaataggcctaggatgcatatggcggccgcttccctttagtgagggttaatgcttcgagcagacatgataagatacattgatgagtttggacaaaccacaactagaatgcagtgaaaaaaatgctttatttgtgaaatttgtgatgctattgctttatttgtaaccattataagctgcaataaacaagttaacaacaacaattgcattcattttatgtttcaggttcagggggagatgtgggaggttttttaaagcaagtaaaacctctacaaatgtggtaaaatccgataaggatcgatccgggctggcgtaatagcgaagaggcccgcaccgatcgcccttcccaacagttgcgcagcctgaatggcgaatggacgcgccctgtagcggcgcattaagcgcggcgggtgtggtggttacgcgcagcgtgaccgctacacttgccagcgccctagcgcccgctcctttcgctttcttcccttcctttctcgccacgttcgcccgatagcgataaggatccgcgtatggtgcactctcagtacaatctgctctgatgccgcatagttaagccagccccgacacccgccaacacccgctgacgcgccctgacgggcttgtctgctcccggcatccgcttacagacaagctgtgaccgtctccgggattttgttactttatagaagaaattttgagtttttgtttttttttaataaataaataaacataaataaattgtttgttgaatttattattagtatgtaagtgtaaatataataaaacttaatatctattcaaattaataaataaacctcgatatacagaccgataaaacacatgcgtcaattttacgcatgattatctttaacgtacgtcacaatatgattatctttctagggttaatccgggagctgcatgtgtcagaggttttcaccgtcatcaccgaaacgcgcgagacgaaagggcctcgtgatacgcctatttttataggttaatgtcatgataataatggtttcttagacgtcaggtggcacttttcggggaaatgtgcgcggaacccctatttgtttatttttctaaatacattcaaatatgtatccgctcatgagacaataaccctgataaatgcttcaataatattgaaaaaggaagagtatgagtattcaacatttccgtgtcgcccttattcccttttttgcggcattttgccttcctgtttttgctcacccagaaacgctggtgaaagtaaaagatgctgaagatcagttgggtgcacgagtgggttacatcgaactggatctcaacagcggtaagatccttgagagttttcgccccgaagaacgttttccaatgatgagcacttttaaagttctgctatgtggcgcggtattatcccgtattgacgccgggcaagagcaactcggtcgccgcatacactattctcagaatgacttggttgagtactcaccagtcacagaaaagcatcttacggatggcatgacagtaagagaattatgcagtgctgccataaccatgagtgataacactgcggccaacttacttctgacaacgatcggaggaccgaaggagctaaccgcttttttgcacaacatgggggatcatgtaactcgccttgatcgttgggaaccggagctgaatgaagccataccaaacgacgagcgtgacaccacgatgcctgtagcaatggcaacaacgttgcgcaaactattaactggcgaactacttactctagcttcccggcaacaattaatagactggatggaggcggataaagttgcaggaccacttctgcgctcggcccttccggctggctggtttattgctgataaatctggagccggtgagcgtgggtctcgcggtatcattgcagcactggggccagatggtaagccctcccgtatcgtagttatctacacgacggggagtcaggcaactatggatgaacgaaatagacagatcgctgagataggtgcctcactgattaagcattggtaactgtcagaccaagtttactcatatatactttagattgatttaaaacttcatttttaatttaaaaggatctaggtgaagatcctttttgataatctcatgaccaaaatcccttaacgtgagttttcgttccactgagcgtcagaccccgtagaaaagatcaaaggatcttcttgagatcctttttttctgcgcgtaatctgctgcttgcaaacaaaaaaaccaccgctaccagcggtggtttgtttgccggatcaagagctaccaactctttttccgaaggtaactggcttcagcagagcgcagataccaaatactgttcttctagtgtagccgtagttaggccaccacttcaagaactctgtagcaccgcctacatacctcgctctgctaatcctgttaccagtggctgctgccagtggcgataagtcgtgtcttaccgggttggactcaagacgatagttaccggataaggcgcagcggtcgggctgaacggggggttcgtgcacacagcccagcttggagcgaacgacctacaccgaactgagatacctacagcgtgagctatgagaaagcgccacgcttcccgaagggagaaaggcggacaggtatccggtaagcggcagggtcggaacaggagagcgcacgagggagcttccagggggaaacgcctggtatctttatagtcctgtcgggtttcgccacctctgacttgagcgtcgatttttgtgatgctcgtcaggggggcggagcctatggaaaaacgccagcaacgcggcctttttacggttcctggccttttgctggccttttgctcacatggctcgacagatctttaaccctagaaagatagtctgcgtaaaattgacgcatgcattcttgaaatattgctctctctttctaaatagcgcgaatccgtcgctgtgcatttaggacatctcagtcgccgcttggagctcccgtgaggcgtgcttgtcaatgcggtaagtgtcactgattttgaactataacgaccgcgtgagtcaaaatgacgcatgattatcttttacgtgacttttaagatttaactcatacgataattatattgttatttcatgttctacttacgtgataacttattatatatatattttcttgttatagataagatcttcaatattggccattagccatattattcattggttatatagcataaatcaatattggctattggccattgcatacgttgtatctatatcataatatgtacatttatattggctcatgtccaatatgaccgccatgttggcattgattattgactagttattaatagtaatcaattacggggtcattagttcatagcccatatatggagttccgcgttacataacttacggtaaatggcccgcctggctgaccgcccaacgacccccgcccattgacgtcaataatgacgtatgttcccatagtaacgccaatagggactttccattgacgtcaatgggtggagtatttacggtaaactgcccacttggcagtacatcaagtgtatcatatgccaagtccgccccctattgacgtcaatgacggtaaatggcccgcctggcattatgcccagtacatgaccttacgggactttcctacttggcagtacatctacgtattagtcatcgctattaccatggtgatgcggttttggcagtacaccaatgggcgtggatagcggtttgactcacggggatttccaagtctccaccccattgacgtcaatgggagtttgttttggcaccaaaatcaacgggactttccaaaatgtcgtaacaactgcgatcgcccgccccgttgacgcaaatgggcggtaggcgtgtacggtgggaggtctatataagcagagctcgtttagtgaaccgtcagatcactagaagctttattgcggtagtttatcacagttaaattgctaacgcagtcagtgcttctgacacaacagtctcgaacttaagctgcagtgactctcttaaggtagccttgcagaagttggtcgtgaggcactgggcaggtaagtatcaaggttacaagacaggtttaaggagaccaatagaaactgggcttgtcgagacagagaagactcttgcgtttctgataggcacctattggtcttactgacatccactttgcctttctctccacaggtgtccactcccagttcaattacagctcttaaggctagagtacttaatacgactcactataggctagcc

SEQ ID NO: 5 - DNA, 681 bp, Homo sapiens
atggctgtgagaagggactccgtgtggaagtactgctggggtgttttgatggttttatgcagaactgcgatttccaaatcgatagttttagagcctatctattggaattcctcgaactccaaatttctacctggacaaggactggtactatacccacagataggagacaaattggatattatttgccccaaagtggactctaaaactgttggccagtatgaatattataaagtttatatggttgataaagaccaagcagacagatgcactattaagaaggaaaatacccctctcctcaactgtgccaaaccagaccaagatatcaaattcaccatcaagtttcaagaattcagccctaacctctggggtctagaatttcagaagaacaaagattattacattatatctacatcaaatgggtctttggagggcctggataaccaggagggaggggtgtgccagacaagagccatgaagatcctcatgaaagttggacaagatgcaagttctgctggatcaaccaggaataaagatccaacaagacgtccagaactagaagctggtacaaatggaagaagttcgacaacaagtccctttgtaaaaccaaatccaggttctagcacagacggcaacagcgccggacattcggggaacaacatcctcggttccgaagtggcctta

SEQ ID NO: 6 - DNA, 15 bp, Artificial Sequence
  linker
tcctcagcggccgca

SEQ ID NO: 7 - DNA, 321 bp, Homo sapiens
attgaagttatgtatcctcctccttacctagacaatgagaagagcaatggaaccattatccatgtgaaagggaaacacctttgtccaagtcccctatttcccggaccttctaagcccttttgggtgctggtggtggttgggggagtcctggcttgctatagcttgctagtaacagtggcctttattattttctgggtgaggagtaagaggagcaggctcctgcacagtgactacatgaacatgactccccgccgccccgggcccacccgcaagcattaccagccctatgccccaccacgcgacttcgcagcctatcgctcc

SEQ ID NO: 8 - DNA, 339 bp, Homo sapiens
agagtgaagttcagcaggagcgcagacgcccccgcgtaccagcagggccagaaccagctctataacgagctcaatctaggacgaagagaggagtacgatgttttggacaagagacgtggccgggaccctgagatggggggaaagccgagaaggaagaaccctcaggaaggcctgtacaatgaactgcagaaagataagatggcggaggcctacagtgagattgggatgaaaggcgagcgccggaggggcaaggggcacgatggcctttaccagggtctcagtacagccaccaaggacacctacgacgcccttcacatgcaggccctgccccctcgctaa

SEQ ID NO: 9 - DNA, 24 bp, Artificial Sequence
  XhoI-EFNB2 forward primer
atctcgagatggctgtgagaaggg

SEQ ID NO: 10 - DNA, 27 bp, Artificial Sequence
  EFNB2 ECD-BbvCI reverse primer
atcctcagcataaggccacttcggaac